European Patent Specification EP 4 019 531 B1, published March 13, 2024. Title: Peptides promoting hair growth and uses thereof. Applicant: CAREGEN CO., LTD. The sequence listing filed with the application follows.

SEQUENCE LISTING (5 sequences)

SEQ ID NO: 1 - protein, 6 aa, Artificial Sequence
  peptide
WQNMRL

SEQ ID NO: 2 - DNA, 21 bp, Artificial Sequence
  TGF beta-1 primer_forward
gccctggataccaactattgc

SEQ ID NO: 3 - DNA, 21 bp, Artificial Sequence
  TGF beta-1 primer_reverse
tcagcacttgcaggagtagcg

SEQ ID NO: 4 - DNA, 25 bp, Artificial Sequence
  GAPDH primer_forward
ggtgtgaacggatttggccgtattg

SEQ ID NO: 5 - DNA, 25 bp, Artificial Sequence
  GAPDH primer_reverse
ccgttgaatttgccgtgagtggagt